European Patent Application EP 4 442 699 A1, published October 9, 2024. Title: CRD.VL THERMOSTABLE PROTEIN DOMAINS WITH LECTIN-LIKE PROPERTIES DERIVED FROM GALECTIN 3. Applicant: UNIVERSITE DE LORRAINE. The sequence listing filed with the application follows.

SEQUENCE LISTING (7 sequences)

SEQ ID NO: 1 - protein, 156 aa, synthetic construct
  VARIANT 28: note = any amino acid
  VARIANT 32: note = any amino acid
  VARIANT 61: note = any amino acid
  VARIANT 100: note = any amino acid
  VARIANT 108: note = any amino acid
  VARIANT 126: note = any amino acid
  VARIANT 128: note = any amino acid
  VARIANT 141: note = any amino acid
MSATGAYPATGPYGAPAGPLIVPYELPXPGGXHPGMLITIQGTVKPNANRIALDFQRGNDXAFHFNPRFNENNRRVIVCNTKQGNQWGPEERQMHFPFEXGKPFKIQXLVEPDHFKVAVNDQHLLXYXHRVKNLQEINKLXISGDIQLTSVSYTMI

SEQ ID NO: 2 - protein, 156 aa, synthetic construct
MSATGAYPATGPYGAPAGPLIVPYELPLPGGVHPGMLITIQGTVKPNANRIALDFQRGNDVAFHFNPRFNENNRRVIVCNTKQGNQWGPEERQMHFPFESGKPFKIQVLVEPDHFKVAVNDQHLLQYNHRVKNLQEINKLGISGDIQLTSVSYTMI

SEQ ID NO: 3 - protein, 156 aa, synthetic construct
MSATGAYPATGPYGAPAGPLIVPYELPLPGGVHPGMLITIQGTVKPNANRIALDFQRGNDVAFHFNPRFNENNRRVIVCNTKQGNQWGPEERQMHFPFERGKPFKIQILVEPDHFKVAVNDQHLLQYNHRVKNLQEINKLRISGDIQLTSVSYTMI

SEQ ID NO: 4 - protein, 156 aa, synthetic construct
MSATGAYPATGPYGAPAGPLIVPYELPIPGGIHPGMLITIQGTVKPNANRIALDFQRGNDIAFHFNPRFNENNRRVIVCNTKQGNQWGPEERQMHFPFERGKPFKIQILVEPDHFKVAVNDQHLLEYKHRVKNLQEINKLRISGDIQLTSVSYTMI

SEQ ID NO: 5 - protein, 156 aa, synthetic construct
  VARIANT 25: note = E or N
  VARIANT 28: note = I or L
  VARIANT 32: note = I or V
  VARIANT 33: note = H or V
  VARIANT 35: note = G or K
  VARIANT 41: note = Q or L
  VARIANT 61: note = I or V
  VARIANT 83: note = Q or L
  VARIANT 84: note = G or D
  VARIANT 86: note = Q or N
  VARIANT 89: note = P or R
  VARIANT 94: note = M or S
  VARIANT 95: note = H or V
  VARIANT 100: note = R or S
  VARIANT 108: note = I or V
  VARIANT 122: note = Q or A
  VARIANT 126: note = E or Q
  VARIANT 128: note = K or N
  VARIANT 133: note = N or K
  VARIANT 135: note = Q or N
  VARIANT 138: note = N or S
  VARIANT 141: note = R or G
  VARIANT 147: note = Q or D
  VARIANT 151: note = V or T
MSATGAYPATGPYGAPAGPLIVPYXLPXPGGXXPXMLITIXGTVKPNANRIALDFQRGNDXAFHFNPRFNENNRRVIVCNTKXXNXWGXEERQXXFPFEXGKPFKIQXLVEPDHFKVAVNDXHLLXYXHRVKXLXEIXKLXISGDIXLTSXSYTMI

SEQ ID NO: 6 - protein, 156 aa, synthetic construct
MSATGAYPATGPYGAPAGPLIVPYNLPLPGGVVPKMLITILGTVKPNANRIALDFQRGNDVAFHFNPRFNENNRRVIVCNTKLDNNWGREERQSVFPFESGKPFKIQVLVEPDHFKVAVNDAHLLQYNHRVKKLNEISKLGISGDIDLTSTSYTMI

SEQ ID NO: 7 - protein, 156 aa, synthetic construct; identical to SEQ ID NO: 1
  VARIANT 28: note = L or I
  VARIANT 32: note = V or I
  VARIANT 61: note = V or I
  VARIANT 100: note = S or R
  VARIANT 108: note = V or I
  VARIANT 126: note = Q or E
  VARIANT 128: note = N or K
  VARIANT 141: note = G or R